European Patent Application EP 4 122 926 A1, published January 25, 2023. Title: TRIAZINE DERIVATIVES HAVING VIRUS PROLIFERATION INHIBITORY ACTION AND PHARMACEUTICAL COMPOSITION CONTAINING THOSE. Applicant: Shionogi & Co., Ltd. NATIONAL UNIVERSITY CORPORATION HOKKAIDO UNIVERSITY. The sequence listing filed with the application follows.

SEQUENCE LISTING (2 sequences)

SEQ ID NO: 1 - protein, 14 aa, Artificial sequence
  Substrate Peptide
EMKRFGSQLVASTK

SEQ ID NO: 2 - protein, 7 aa, Artificial sequence
  Internal Standard Peptide
QLVASTK